European Patent Application EP 4 477 663 A1, published December 18, 2024. Title: Novel proteins for isothermal amplification. Applicant: midge medical GmbH. Application EP. The sequence listing filed with the application follows.

SEQUENCE LISTING (20 sequences)

SEQ ID NO: 1 - protein, 306 aa, Lutimaribacter sp. EGI FJ00015
MFKRKNPAALASQLASLSGSKGFNSEDKGEWKLKLDNAGNGQAVIRFLPGKGDEGVPFAVLVNHGFKKGGKWYIENCTSTHGDYDSCPVCQYLSKNDSYNTNNEEYKLLKRKTSYYANILVVKDPAAPENEGKVFKYRFGKKIWDKINAMVAVDVEMGETPIDVTCAFEGANFVLKVKKVSGFSNYDESKFLGQSEIPNIEDEAYQAQLQEQMVDLSTLTAKDQFKSFEDNQKKFLQVMGTAAMGTAASRASAQADKVGEDLDNFEDDLASFNAGSQKSAPAEDFMETGGSASSGDEDLDELLNGL

SEQ ID NO: 2 - protein, 164 aa, Lutimaribacter sp. EGI FJ00015
MAGSVNKVILVGNLGRDPEVRTFQNGGRVCNLRIATSENWKDRNTGERRERTEWHSVAIFNENLARLAEQYLRKGSKVYVEGKLETRKWQDQSGQDRYSTEVVLRPYAGELTFLDSRDSGGGGGGGGSQGGGYDSGGDYGGGYDSGPGSSAPAPSRDLDDEIPF

SEQ ID NO: 3 - protein, 301 aa, Shigella flexneri
MFKRKSTAELAAQMAKLNGNKGFSSEDKGEWKLKLDNAGNGQAVIRFLPSKNDEQAPFAILVNHGFKKNGKWYIETCSSTHGDYDSCPVCQYISKNDLYNTDNKEYSLVKRKTSYWANILVVKDPAAPENEGKVFKYRFGKKIWDKINAMIAVDVEMGETPVDVTCPWEGANFVLKVKQVSGFSNYDESKFLNQSAIPNIDDESFQKELFEQMVDLSEMTSKDKFKSFEELNTKFGQVMGTAVMGGAAATAAKKADKVTDDLDAFNVDDFKTKTEDDFMSSSSGSSSGADDTDLDDLLNDL

SEQ ID NO: 4 - protein, 261 aa, Escherichia phage lambda
MSTALATLAGKLAERVGMDSVDPQELITTLRQTAFKGDASDAQFIALLIVANQYGLNPWTKEIYAFPDKQNGIVPVVGVDGWSRIINENQQFDGMDFEQDNESCTCRIYRKDRNHPICVTEWMDECRREPFKTREGREITGPWQSHPKRMLRHKAMIQCARLAFGFAGIYDKDEAERIVENTAYTAERQPERDITPVNDETMQEINTLLIALDKTWDDDLLPLCSQIFRRDIRASSELTQAEAVKALGFLKQKAAEQKVAA

SEQ ID NO: 5 - protein, 387 aa, Lutimaribacter sp. EGI FJ00015
MSDLKSRLIKASTSKMTASLDKSKFFNEKDVVRTKIPMLNIAISGALDGGMQSGLTIFAGPSKHFKSNMSLTMVSAYMTKYPDAICLFYDSEFGITPAYLRAMGVDPDRVVHTPVQSVEQLKIDMVNQLEEIERGEKVIVFIDSIGNLAYKKETEDALNEKSVADMTRAKSLKSLFRIVTPYFSIKNIPCVAVNHTIETIEMFSKTVMTGGTGPMYSADTVFIIGKRQIKDGTDLQGYQFVLNAEKSRTVKEKSKFFIDVKFDGGIDPYSGLLDMALELGFVVKPKNGWYAREYLDVDTGEMVREEKSWRAKDTSSTAFWGPLFKHQPFRDAIKNRYQLGAIETNAVVDEEVDALINSKTEEFHAPEGEVRATPASIEDELENYDEE

SEQ ID NO: 6 - protein, 387 aa, Lutimaribacter sp. EGI FJ00015
MSDLKSRLIKASTSKMTASLDKSKFFNEKDVVRTKIPMLNIAISGALDGGMQSGLTIFAGPSKSFKSNMSLTMVSAYMTKYPDAICLFYDSEFGITPAYLRAMGVDPDRVVHTPVQSVEQLKIDMVNQLEEIERGEKVIVFIDSIGNLAYKKETEDALNEKSVADMTRAKSLKSLFRIVTPYFSIKNIPCVAVNHTIETIEMFSKTVMTGGTGPMYSADTVFIIGKRQIKDGTDLQGYQFVLNAEKSRTVKEKSKFFIDVKFDGGIDPYSGLLDMALELGFVVKPKNGWYAREYLDVDTGEMVREEKSWRAKDTSSTAFWGPLFKHQPFRDAIKNRYQLGAIETNAVVDEEVDALINSKTEEFHAPEGEVRATPASIEDELENYDEE

SEQ ID NO: 7 - protein, 350 aa, Lutimaribacter sp. EGI FJ00015
MDSKKNADKQKALDSALAQIERQFGKGSIMKMGSDNPVRDIEATSTGSLGLDIALGIGGLPKGRIIEIYGPESSGKTTLTLHCIAEEQKKGGVSAFVDAEHAFDPQYAKKLGVDLDELLISQPDTGEQALEIVDTLVRSGAVNMVVVDSVAALTPKSELEGDMGDSSVGVQARLMSQAMRKLTGSISRSNCMVIFINQIRMKIGVMFGSPETTTGGNALKFYSSVRLDIRRIGSVKDRDEVVGNATRVKVAKNKVAPPFKQVEFDIMYGEGISKMGEILDLGVKAGVVDKSGAWYSYGDERIGQGRENAKTFLRENAAMALEIEDKIRAAHGLDFAMSDDTPDDSEVFEG

SEQ ID NO: 8 - protein, 390 aa, Shigella flexneri
MSDLKSRLIKASTSKMTADLTKSKLFNNRDEVPTRIPMLNIALGGALNAGLQSGLTIFAAPSKHFKTLFGLTMVAAYMKKYKDAICLFYDSEFGASESYFRSMGVDLDRVVHTPIQSVEQLKVDMTNQLDAIERGDKVIIFIDSIGNTASKKETEDALNEKVVGDMSRAKALKSLFRIVTPYLTIKDIPCVAINHTAMEIGGLYPKEIMGGGTGILYSANTVFFISKRQVKEGTELTGYDFTLKAEKSRTVKEKSTFPITVNFDGGIDPFSGLLEMATEIGFVVKPKAGWYAREFLDEETGEMIREEKSWRAKATDCVEFWGPLFKHKPFRDAIETKYKLGAISSIKEVDDAVNDLINCKATTKVPVKASDAPSAADIENDLDEMEDFDE

SEQ ID NO: 9 - protein, 269 aa, Escherichia coli
MTKQPPIAKADLQKTQGNRAPAAVKNSDVISFINQPSMKEQLAAALPRHMTAERMIRIATTEIRKVPALGNCDTMSFVSAIVQCSQLGLEPGSALGHAYLLPFGNKNEKSGKKNVQLIIGYRGMIDLARRSGQIASLSARVVREGDEFSFEFGLDEKLIHRPGENEDAPVTHVYAVARLKDGGTQFEVMTRKQIELVRSLSKAGNNGPWVTHWEEMAKKTAIRRLFKYLPVSIEIQRAVSMDEKEPLTIDPADSSVLTGEYSVIDNSEE

SEQ ID NO: 10 - protein, 146 aa, Escherichia phage lambda
MKKLTFEIRSPAHQQNAIHAVQQILPDPTKPIVVTIQERNRSLDQNRKLWACLGDVSRQVEWHGRWLDAESWKCVFTAALKQQDVVPNLAGNGFVVIGQSTSRMRVGEFAELLELIQAFGTERGVKWSDEARLALEWKARWGDRAA

SEQ ID NO: 11 - DNA, 921 bp, Lutimaribacter sp. EGI FJ00015
  source 1..921: mol_type = other DNA
atgtttaagcgtaaaaatcctgctgccctggcttcccaactggcttccctgtctggttctaaaggtttcaattccgaagataaaggtgaatggaaactgaagttggataatgctggtaacggtcaagcggtcatccgtttcctgccaggtaaaggtgatgaaggcgtaccattcgctgttctagtgaatcacggcttcaagaaaggtggtaaatggtacattgaaaactgtacttctacccacggtgattatgattcttgcccagtatgtcaatatctgtccaagaatgattcatataacaccaacaatgaagaatacaagctgttgaaacgcaaaacttcttactacgcgaacatcctggttgttaaagaccctgctgctccagaaaacgaaggtaaagtcttcaaatatcgtttcggtaagaaaatttgggacaaaatcaatgcaatggttgccgttgacgttgaaatgggcgaaactccaatcgacgtaacttgtgcgtttgaaggtgctaacttcgttctgaaagttaagaaagtatctggtttcagcaactatgatgaatccaagttccttggccaatctgagattcctaacatcgaagatgaagcttatcaagcacagctgcaggaacaaatggttgacctgtctactctgactgcgaaagaccagttcaaatctttcgaagataaccagaagaaattccttcaggttatgggtacagctgctatgggtactgccgcgtctcgcgcttctgcccaggctgataaggttggtgaagacctggacaactttgaagatgacctcgcgagctttaacgcaggttctcagaaatcagcaccagctgaagacttcatggaaactggcggttctgcctccagcggtgatgaagacctagacgaactgctgaacggtctgtaa

SEQ ID NO: 12 - DNA, 495 bp, Lutimaribacter sp. EGI FJ00015
  source 1..495: mol_type = other DNA
atggctggctcggtgaacaaggtaattctggtgggcaacctggggcgcgaccccgaggtgcgcacattccagaacgggggacgcgtatgcaacctgcgcatcgccacatcggaaaactggaaagaccgcaacaccggcgagcggcgcgaacggaccgagtggcactcggtcgccatcttcaatgaaaaccttgcccgactggccgaacaatacctgcgcaaggggtccaaggtctatgtcgagggcaagctggaaacccggaaatggcaagaccagtcgggccaggaccgctactcgaccgaggtcgtgctgcgcccctatgccggcgagctgacctttctcgacagccgcgacagcggcggcggcggtggtggtggcgggagccagggcggtggctatgacagcggcggtgattacggtggcggctatgacagcggccccggcagcagcgcgcccgccccgtcacgcgacctggacgacgagatcccgttctga

SEQ ID NO: 13 - DNA, 906 bp, Shigella flexneri
  source 1..906: mol_type = other DNA
atgtttaaacgtaaatctactgctgaacttgctgcacaaatggctaaactgaatggcaataaaggtttttcttctgaagataaaggcgagtggaaactgaaactcgataatgcgggtaacggtcaagcagtaattcgttttcttccgtctaaaaatgatgaacaagcaccattcgcaattcttgtaaatcacggtttcaagaaaaatggtaaatggtatattgaaacatgttcatctacccacggtgattacgattcttgcccagtatgtcaatacatcagtaaaaatgatctgtacaacactgacaataaagagtacagtcttgttaaacgtaaaacttcttactgggctaacattcttgtagtaaaagacccagctgctccagaaaacgaaggtaaagtatttaaataccgtttcggtaagaaaatctgggataaaatcaacgcgatgattgcagttgatgtcgaaatgggtgaaactccggttgatgtaacttgtccgtgggaaggtgctaactttgtactgaaagttaaacaagtttccggatttagtaactacgacgaatctaaattcctgaatcaatctgcgattccaaacattgacgatgaatctttccagaaagaactgttcgaacaaatggttgacctttctgaaatgacttctaaagataaattcaaatcgtttgaagaactgaatactaaattcggtcaagttatgggaactgctgtgatgggcggtgccgcagcaactgccgctaagaaagctgataaagttactgatgatttggatgcattcaatgttgatgacttcaaaacaaaaactgaagatgattttatgagctcaagctctggcagttcatctggtgctgatgacacggacctggatgaccttttgaatgacctttaa

SEQ ID NO: 14 - DNA, 786 bp, Escherichia phage lambda
  source 1..786: mol_type = other DNA
atgagtactgcactcgcaacgctggctgggaagctggctgaacgtgtcggcatggattctgtcgacccacaggaactgatcaccactcttcgccagacggcatttaaaggtgatgccagcgatgcgcagttcatcgcattactgatcgttgccaaccagtacggccttaatccgtggacgaaagaaatttacgcctttcctgataagcagaatggcatcgttccggtggtgggcgttgatggctggtcccgcatcatcaatgaaaaccagcagtttgatggcatggactttgagcaggacaatgaatcctgtacatgccggatttaccgcaaggaccgtaatcatccgatctgcgttaccgaatggatggatgaatgccgccgcgaaccattcaaaactcgcgaaggcagagaaatcacggggccgtggcagtcgcatcccaaacggatgttacgtcataaagccatgattcagtgtgcccgtctggccttcggatttgctggtatctatgacaaggatgaagccgagcgcattgtcgaaaatactgcatacactgcagaacgtcagccggaacgcgacatcactccggttaacgatgaaaccatgcaggagattaacactctgctgatcgccctggataaaacatgggatgacgacttattgccgctctgttcccagatatttcgccgcgacattcgtgcatcgtcagaactgacacaggccgaagcagtaaaagctcttggattcctgaaacagaaagccgcagagcagaaggtggcagcatga

SEQ ID NO: 15 - DNA, 1164 bp, Lutimaribacter sp. EGI FJ00015
  source 1..1164: mol_type = other DNA
atgtctgatttaaaatctcgtctgattaaagcatccacttctaaaatgaccgcatctctggataaatccaaattcttcaatgaaaaggatgtagttcgtactaagattccgatgcttaatatcgcgatttcaggtgcattagatggtggcatgcaatcaggtttaacaatctttgcgggcccgtcaaagcacttcaagtcaaatatgagtctgactatggtttccgcttatatgacaaaatatccggatgctatttgtctgttctacgactcagaattcggtatcactccagcatatcttcgtgcaatgggtgttgacccggaccgtgtagtacacactcctgtacaatctgttgagcagcttaagattgacatggtcaaccagctggaagaaattgaacgcggtgagaaagttatcgtattcatcgactccatcggtaaccttgcttataagaaagaaacagaagatgctctgaacgaaaaatcagttgcggatatgactcgtgcgaaatcactgaagtctctgttccgtattgttacaccttacttctctatcaaaaacattccatgcgttgcggttaaccacacaatcgaaacaattgagatgttcagtaagactgtaatgactggtggtactggcccaatgtattcagcagatactgtgttcatcattggtaaacgtcaaattaaagatggtacagaccttcaaggttatcagtttgttctgaatgctgagaaatctcgtactgttaaagagaagagtaagttcttcattgatgttaaattcgatggcggtattgacccatactctggtctgttggatatggcgctggaacttggttttgtagttaaacctaaaaacggttggtatgctcgtgaatatctggacgtagataccggtgaaatggttcgcgaagagaaatcatggcgtgcaaaagatacttcaagcaccgcattttggggccctctgtttaaacatcagccattccgcgatgctattaaaaatcgctatcagctgggtgctattgaaaccaatgcagtagtagatgaagaagttgatgctctgattaattcgaagaccgaagagttccatgctccggaaggcgaagtaagagcaactccagcttcaatcgaagatgaactggaaaattacgatgaagaataa

SEQ ID NO: 16 - DNA, 1164 bp, Lutimaribacter sp. EGI FJ00015
  source 1..1164: mol_type = other DNA
atgtctgatttaaaatctcgtctgattaaagcatccacttctaaaatgaccgcatctctggataaatccaaattcttcaatgaaaaggatgtagttcgtactaagattccgatgcttaatatcgcgatttcaggtgcattagatggtggcatgcaatcaggtttaacaatctttgcgggcccgtcaaagtcattcaagtcaaatatgagtctgactatggtttccgcttatatgacaaaatatccggatgctatttgtctgttctacgactcagaattcggtatcactccagcatatcttcgtgcaatgggtgttgacccggaccgtgtagtacacactcctgtacaatctgttgagcagcttaagattgacatggtcaaccagctggaagaaattgaacgcggtgagaaagttatcgtattcatcgactccatcggtaaccttgcttataagaaagaaacagaagatgctctgaacgaaaaatcagttgcggatatgactcgtgcgaaatcactgaagtctctgttccgtattgttacaccttacttctctatcaaaaacattccatgcgttgcggttaaccacacaatcgaaacaattgagatgttcagtaagactgtaatgactggtggtactggcccaatgtattcagcagatactgtgttcatcattggtaaacgtcaaattaaagatggtacagaccttcaaggttatcagtttgttctgaatgctgagaaatctcgtactgttaaagagaagagtaagttcttcattgatgttaaattcgatggcggtattgacccatactctggtctgttggatatggcgctggaacttggttttgtagttaaacctaaaaacggttggtatgctcgtgaatatctggacgtagataccggtgaaatggttcgcgaagagaaatcatggcgtgcaaaagatacttcaagcaccgcattttggggccctctgtttaaacatcagccattccgcgatgctattaaaaatcgctatcagctgggtgctattgaaaccaatgcagtagtagatgaagaagttgatgctctgattaattcgaagaccgaagagttccatgctccggaaggcgaagtaagagcaactccagcttcaatcgaagatgaactggaaaattacgatgaagaataa

SEQ ID NO: 17 - DNA, 1053 bp, Lutimaribacter sp. EGI FJ00015
  source 1..1053: mol_type = other DNA
atggacagcaaaaaaaacgccgacaagcaaaaggcgctagacagcgctctggcccagatcgaacggcagttcggcaaggggtcgatcatgaagatgggcagcgacaacccggttcgggatatcgaggcaacatcgaccggctccctggggctggatatcgcgctgggcatcggcgggctgcccaaggggcggatcatcgagatctacgggcccgaatcctccggcaagacgacgttgaccctgcactgcatcgcggaagagcagaagaaaggcggcgtttccgcctttgtcgatgccgaacacgcctttgacccgcaatacgccaagaaactgggcgttgacctggacgaactgctgatcagccagcccgacaccggcgaacaggcgctggagatcgtggatacgcttgtgcgctcgggcgcggtgaacatggtggtggtcgactcggtcgcggcgctgaccccgaagtccgagcttgaaggcgatatgggcgacagcagcgtgggcgtgcaggcccgcctgatgagccaggcaatgcgcaagttgaccggctcgatcagccgctcgaactgcatggttattttcatcaaccagatccggatgaagattggcgtgatgttcggcagccccgaaaccaccaccggcggcaacgccctgaaattctacagctcggtccggctggatattcgccggatcggatcggtcaaggaccgtgacgaggtggtcggtaacgcgacccgcgtgaaagtggccaagaacaaggtggcgccgccgttcaagcaggtcgagttcgacatcatgtacggcgaaggcatctcgaagatgggcgaaatcctggatcttggcgtcaaggccggcgtggtcgacaaatccggcgcctggtacagctacggcgacgagcggatcgggcaggggcgcgagaacgccaagaccttcctgcgcgaaaacgcggccatggcgctggagatcgaggacaagatccgcgcggcgcacgggctggatttcgccatgtccgacgatacgccggatgacagcgaggtgttcgagggctga

SEQ ID NO: 18 - DNA, 1173 bp, Shigella flexneri
  source 1..1173: mol_type = other DNA
atgtctgatttaaaatctcgtctgattaaagcttctacttctaaaatgactgcagacttgactaagtctaagctgtttaataatcgtgatgaagtccctactcgtattccgatgttgaatatcgcactaggtggtgctctgaatgcaggattgcaatcaggcttgactatttttgctgcaccttctaaacattttaaaacattgtttgggctgactatggttgcagcgtatatgaagaaatataaagatgcaatctgtttgttttatgactcggaatttggtgcttcagaatcttattttcgttcaatgggtgttgatttagaccgtgtagttcatactccgattcaatctgtcgaacaacttaaagttgatatgactaatcagcttgacgctattgaacgcggtgataaagttattatctttatcgattcaatcggtaatactgcatctaagaaagaaaccgaagatgcattgaacgagaaagtcgtaggtgatatgtctcgtgctaaggcacttaaatctctgttccgtattgtgaccccgtatctgactattaaagatattccatgtgttgcaatcaaccatacagcaatggaaatcggcggactatatcctaaagagattatgggtggtggtacaggtattctttactctgctaacactgtattctttatctctaaacgtcaggttaaagaaggtacagaattgaccggttatgacttcacgttgaaagcagaaaaatctcgtacagttaaagagaaatctactttcccaatcacggttaattttgatggcggtattgatccattcagtggcttgttagaaatggcaactgaaattggatttgttgttaagcctaaagctggttggtatgctcgtgaattccttgacgaagaaacaggtgaaatgattcgtgaagaaaaatcatggcgtgctaaagctactgattgtgtagaattctggggaccgttgtttaaacacaaacctttccgagatgcaattgaaactaaatataaactaggtgctatctcttctattaaagaagttgatgacgctgttaacgaccttattaattgcaaagcaacaactaaagttcctgttaaagcttctgatgctccgtctgcagcagatatagaaaacgaccttgacgaaatggaagatttcgatgaataa

SEQ ID NO: 19 - DNA, 810 bp, Escherichia coli
  source 1..810: mol_type = other DNA
atgactaagcaaccaccaatcgcaaaagccgatctgcaaaaaactcagggaaaccgtgcaccagcagcagttaaaaatagcgacgtgattagttttattaaccagccatcaatgaaagagcaactggcagcagctcttccacgccatatgacggctgaacgtatgatccgtatcgccaccacagaaattcgtaaagttccggcgttaggaaactgtgacactatgagttttgtcagtgcgatcgtacagtgttcacagctcggacttgagccaggtagcgccctcggtcatgcatatttactgccttttggtaataaaaacgaaaagagcggtaaaaagaacgttcagctaatcattggctatcgcggcatgattgatctggctcgccgttctggtcaaatcgccagcctgtcagcccgtgttgtccgtgaaggtgacgagtttagcttcgaatttggccttgatgaaaagttaatacaccgcccgggagaaaacgaagatgccccggttacccacgtctatgctgtcgcaagactgaaagacggaggtactcagtttgaagttatgacgcgcaaacagattgagctggtgcgcagcctgagtaaagctggtaataacgggccgtgggtaactcactgggaagaaatggcaaagaaaacggctattcgtcgcctgttcaaatatttgcccgtatcaattgagatccagcgtgcagtatcaatggatgaaaaggaaccactgacaatcgatcctgcagattcctctgtattaaccggggaatacagtgtaatcgataattcagaggaataa

SEQ ID NO: 20 - DNA, 441 bp, Escherichia phage lambda
  source 1..441: mol_type = other DNA
atgaaaaaactaacctttgaaattcgatctccagcacatcagcaaaacgctattcacgcagtacagcaaatccttccagacccaaccaaaccaatcgtagtaaccattcaggaacgcaaccgcagcttagaccaaaacaggaagctatgggcctgcttaggtgacgtctctcgtcaggttgaatggcatggtcgctggctggatgcagaaagctggaagtgtgtgtttaccgcagcattaaagcagcaggatgttgttcctaaccttgccgggaatggctttgtggtaataggccagtcaaccagcaggatgcgtgtaggcgaatttgcggagctattagagcttatacaggcattcggtacagagcgtggcgttaagtggtcagacgaagcgagactggctctggagtggaaagcgagatggggagacagggctgcatga